European Patent Specification EP 3 522 944 B1, published April 3, 2024. Title: A bone implant. Applicant: Ollila, Fredrik Lindfors, Nina Bjorkenheim, Robert Stromberg, Gustav Hupa, Leena Uppstu, Peter Pajarinen, Jukka. The sequence listing filed with the application follows.

SEQUENCE LISTING (6 sequences)

SEQ ID NO: 1 - DNA, 20 bp, Artificial Sequence
  primer
cacccatggcagaagaagga

SEQ ID NO: 2 - DNA, 20 bp, Artificial Sequence
  primer
atccgcatgatctgcatggt

SEQ ID NO: 3 - DNA, 20 bp, Artificial Sequence
  primer
gagtccccaaacaacctcca

SEQ ID NO: 4 - DNA, 20 bp, Artificial Sequence
  primer
tgagtgaggagcacgtagga

SEQ ID NO: 5 - DNA, 20 bp, Artificial Sequence
  primer
cgagctgaacgggaaactca

SEQ ID NO: 6 - DNA, 20 bp, Artificial Sequence
  primer
tgggtggcactgttgaagtc